European Patent Application EP 4 268 843 A2, published November 1, 2023. Title: IMPROVED IL-6 ANTIBODIES. Applicant: F. Hoffmann-La Roche Ltd. Application EP, filed November 6, 2015. The sequence listing filed with the application follows.

SEQUENCE LISTING (54 sequences)

SEQ ID NO: 1 - protein, 225 aa, synthetic construct
QVQLVQSGAEVKKPGSSVKVSCKASGYALSNYLIEWVRQAPGQGLEWMGVITPGSGTINYAQKFQGRVTITADESTSTAYMELSSLRSEDTAVYYCARSRWDPLYYYALEYWGQGTTVTVSSASTKGPSVFPLAPSSKSTSGGTAALGCLVKDYFPEPVTVSWNSGALTSGVHTFPAVLQSSGLYSLSSVVTVPSSSLGTQTYICNVNHKPSNTKVDKKVEPKSC

SEQ ID NO: 2 - protein, 218 aa, synthetic construct
DIVMTQSPDSLAVSLGERATINCRASESVDNYGIPFMNWYQQKPGQPPKLLIYAASNRGSGVPDRFSGSGSGTDFTLTISSLQAEDVAVYYCQQSEEVPLTFGQGTKLEIKRTVAAPSVFIFPPSDEQLKSGTASVVCLLNNFYPREAKVQWKVDNALQSGNSQESVTEQDSKDSTYSLSSTLTLSKADYEKHKVYACEVTHQGLSSPVTKSFNRGEC

SEQ ID NO: 3 - protein, 225 aa, synthetic construct
QVQLVQSGAEVKKPGSSVKVSCKASGYALSNYLIEWVRQAPGQGLEWMGVITPGSGTINYAQKFQGRVTITADESTSTVYMELSSLRSEDTAVYYCARSRWDPLYYYALEYWGQGTTVTVSSASTKGPSVFPLAPSSKSTSGGTAALGCLVKDYFPEPVTVSWNSGALTSGVHTFPAVLQSSGLYSLSSVVTVPSSSLGTQTYICNVNHKPSNTKVDKKVEPKSC

SEQ ID NO: 4 - protein, 10 aa, synthetic construct
GYALSNYLIE

SEQ ID NO: 5 - protein, 10 aa, synthetic construct
VITPGSGTIN

SEQ ID NO: 6 - protein, 13 aa, synthetic construct
SRWDPLYYYALEY

SEQ ID NO: 7 - protein, 15 aa, synthetic construct
RASESVDNYGIPFMN

SEQ ID NO: 8 - protein, 7 aa, synthetic construct
AASNRGS

SEQ ID NO: 9 - protein, 9 aa, synthetic construct
QQSEEVPLT

SEQ ID NO: 10 - protein, 448 aa, synthetic construct
QVQLVQSGAEVKKPGSSVKVSCKASGYALSNYLIEWVRQAPGQGLEWMGVITPGSGTINYAQKFQGRVTITADESTSTAYMELSSLRSEDTAVYYCARSRWDPLYYYALEYWGQGTTVTVSSASTKGPSVFPLAPCSRSTSESTAALGCLVKDYFPEPVTVSWNSGALTSGVHTFPAVLQSSGLYSLSSVVTVPSSNFGTQTYTCNVDHKPSNTKVDKTVERKCCVECPPCPAPPVAGPSVFLFPPKPKDTLMISRTPEVTCVVVDVSHEDPEVQFNWYVDGVEVHNAKTKPREEQFNSTFRVVSVLTVVAQDWLNGKEYKCKVSNKGLPAPIEKTISKTKGQPREPQVYTLPPSREEMTKNQVSLTCLVKGFYPSDIAVEWESNGQPENNYKTTPPMLDSDGSFFLYSKLTVDKSRWQQGNVFSCSVMHEALHNHYTQKSLSLSPGK

SEQ ID NO: 11 - protein, 448 aa, synthetic construct
QVQLVQSGAEVKKPGSSVKVSCKASGYALSNYLIEWVRQAPGQGLEWMGVITPGSGTINYAQKFQGRVTITADESTSTAYMELSSLRSEDTAVYYCARSRWDPLYYYALEYWGQGTTVTVSSASTKGPSVFPLAPCSRSTSESTAALGCLVKDYFPEPVTVSWNSGALTSGVHTFPAVLQSSGLYSLSSVVTVPSSNFGTQTYTCNVDHKPSNTKVDKTVERKCCVECPPCPAPPVAGPSVFLFPPKPKDTLMISRTPEVTCVVVDVSHEDPEVQFNWYVDGVEVHNAKTKPREEQFNSTFRVVSVLTVVHQDWLNGKEYKCKVSNKGLPAPIEKTISKTKGQPREPQVYTLPPSREEMTKNQVSLTCLVKGFYPSDIAVEWESNGQPENNYKTTPPMLDSDGSFFLYSKLTVDKSRWQQGNVFSCSVMHEALHNHYTQKSLSLSPGK

SEQ ID NO: 12 - protein, 218 aa, synthetic construct; identical to SEQ ID NO: 2

SEQ ID NO: 13 - protein, 122 aa, Mus sp.
QVQLQQSGAELVRPGTSVKVSCKASGYAFSNYLIEWVKQRPGQGLEWIGVITPGSGTINYNEKFKGKAVLTADKSSSTVYMQLSSLTSDDSAVYFCAKSRWDPLYYYALEYWGQGTSVTVSS

SEQ ID NO: 14 - protein, 111 aa, Mus sp.
DIVLTQSPASLAVSLGQRATISCRASESVDNYGISFMNWFQQKPGQPPKLLIYAASNQGSGVPARFSGSGSGTDFSLNIHPMEEDDTAMYFCQQSKEVPLTFGAGTKLELK

SEQ ID NO: 15 - protein, 122 aa, synthetic construct
QVQLVQSGAEVKKPGSSVKVSCKASGYAFSNYLIEWVRQAPGQGLEWMGVITPGSGTINYAQKFQGRVTITADESTSTAYMELSSLRSEDTAVYYCARSRWDPLYYYALEYWGQGTTVTVSS

SEQ ID NO: 16 - protein, 111 aa, synthetic construct
DIVMTQSPDSLAVSLGERATINCRASESVDNYGISFMNWYQQKPGQPPKLLIYAASNQGSGVPDRFSGSGSGTDFTLTISSLQAEDVAVYYCQQSKEVPLTFGQGTKLEIK

SEQ ID NO: 17 - protein, 122 aa, synthetic construct
QVQLVQSGAEVKKPGSSVKVSCKASGYALSNYLIEWVRQAPGQGLEWMGVITPGSGTINYAQKFQGRVTITADESTSTAYMELSSLRSEDTAVYYCARSRWDPLYYYALEYWGQGTTVTVSS

SEQ ID NO: 18 - protein, 114 aa, synthetic construct
DIVMTQSPDSLAVSLGERATINCRASESVDNYGIPFMNWYQQKPGQPPKLLIYAASNRGSGVPDRFSGSGSGTDFTLTISSLQAEDVAVYYCQQSEEVPLTFGQGTKLEIKRTV

SEQ ID NO: 19 - protein, 452 aa, synthetic construct
QVQLVQSGAEVKKPGSSVKVSCKASGYALSNYLIEWVRQAPGQGLEWMGVITPGSGTINYAQKFQGRVTITADESTSTAYMELSSLRSEDTAVYYCARSRWDPLYYYALEYWGQGTTVTVSSASTKGPSVFPLAPSSKSTSGGTAALGCLVKDYFPEPVTVSWNSGALTSGVHTFPAVLQSSGLYSLSSVVTVPSSSLGTQTYICNVNHKPSNTKVDKKVEPKSCDKTHTCPPCPAPELLGGPSVFLFPPKPKDTLMISRTPEVTCVVVDVSHEDPEVKFNWYVDGVEVHNAKTKPREEQYNSTYRVVSVLTVLHQDWLNGKEYKCKVSNKALPAPIEKTISKAKGQPREPQVYTLPPSRDELTKNQVSLTCLVKGFYPSDIAVEWESNGQPENNYKTTPPVLDSDGSFFLYSKLTVDKSRWQQGNVFSCSVMHEALHNHYTQKSLSLSPGK

SEQ ID NO: 20 - DNA, 1356 bp, synthetic construct
  source 1..1356: mol_type = other DNA
caagtgcagctggtgcagtcaggggccgaggttaagaagccagggagcagcgtcaaggtatcttgtaaagcgtctggttacgccctttcaaactacctgatcgaatgggtgaggcaggctcccggccaaggcctggaatggatgggagttatcacccctgggagcggcaccattaattacgcccagaaatttcagggacgagtgacgattaccgccgacgagtccaccagtactgcctacatggagctgtcctcactccgcagcgaggacacggcagtttactactgcgcccggagtcgatgggaccctctttactattatgctctggaatactggggccagggaacgaccgttacagtgtcatctgctagcacaaaaggaccatcagtcttcccacttgctccttcatctaagagcacaagtggtggcactgcagcccttggctgcctggtgaaagattatttccccgaacctgttacagtttcttggaactccggtgcactgacatccggagtacacactttcccagctgtgctgcagagctcaggactgtatagcctgtcttcggtggtcactgttccatcgtcgagtcttggcacacagacatatatttgcaacgtcaatcacaagccctccaacacaaaagtggataagaaggtcgagcccaaatcttgtgacaagacccatacgtgtcctccctgtcccgcccctgaactgctgggaggcccttctgtgttcctgttcccacctaagccaaaggacactctgatgatcagccggactcccgaggttacctgtgtggtggtggatgtgtctcatgaagaccctgaggttaagttcaattggtacgtggatggcgtcgaggtgcataacgcaaaaaccaagccgagagaggagcagtacaatagcacctatagagtagtgagcgtcctgactgtcttacatcaggattggctcaatggtaaagaatataagtgcaaggtaagcaacaaggccctacccgcaccaatagagaagaccatctccaaggcgaaaggtcagcccagggagccccaggtttatacactgcctccctcacgcgacgaattaacaaagaatcaggtgtctctcacctgtctcgtcaagggcttttacccttccgacatcgccgtggagtgggaatccaatggccagcctgagaacaattataagacaactcccccagtcctggattcagatgggtcgttctttctatatagtaagttgaccgtggataagtctcgctggcaacaggggaacgtgttctcttgctctgttatgcatgaagcgctgcacaatcattatacccagaagtccctgtccctgagccccgggaag

SEQ ID NO: 21 - protein, 212 aa, Homo sapiens
MNSFSTSAFGPVAFSLGLLLVLPAAFPAPVPPGEDSKDVAAPHRQPLTSSERIDKQIRYILDGISALRKETCNKSNMCESSKEALAENNLNLPKMAEKDGCFQSGFNEETCLVKIITGLLEFEVYLEYLQNRFESSEEQARAVQMSTKVLIQFLQKKAKNLDAITTPDPTTNASLLTKLQAQNQWLQDMTTHLILRSFKEFLQSSLRALRQM

SEQ ID NO: 22 - protein, 218 aa, synthetic construct; identical to SEQ ID NO: 2

SEQ ID NO: 23 - protein, 448 aa, synthetic construct; identical to SEQ ID NO: 11

SEQ ID NO: 24 - protein, 230 aa, synthetic construct
QVQLVQSGAEVKKPGSSVKVSCKASGYALSNYLIEWVRQAPGQGLEWMGVITPGSGTINYAQKFQGRVTITADESTSTAYMELSSLRSEDTAVYYCARSRWDPLYYYALEYWGQGTTVTVSSASTKGPSVFPLAPSSKSTSGGTAALGCLVKDYFPEPVTVSWNSGALTSGVHTFPAVLQSSGLYSLSSVVTVPSSSLGTQTYICNVNHKPSNTKVDKKVEPKSCDKTHT

SEQ ID NO: 25 - protein, 327 aa, synthetic construct
SASTKGPSVFPLAPCSRSTSESTAALGCLVKDYFPEPVTVSWNSGALTSGVHTFPAVLQSSGLYSLSSVVTVPSSNFGTQTYTCNVDHKPSNTKVDKTVERKCCVECPPCPAPPVAGPSVFLFPPKPKDTLMISRTPEVTCVVVDVSHEDPEVQFNWYVDGVEVHNAKTKPREEQFNSTFRVVSVLTVVHQDWLNGKEYKCKVSNKGLPAPIEKTISKTKGQPREPQVYTLPPSREEMTKNQVSLTCLVKGFYPSDIAVEWESNGQPENNYKTTPPMLDSDGSFFLYSKLTVDKSRWQQGNVFSCSVMHEALHNHYTQKSLSLSPGK

SEQ ID NO: 26 - DNA, 654 bp, synthetic construct
  source 1..654: mol_type = other DNA
gacatagtgatgactcaaagtccggacagcctggcggtgtcactcggcgaacgggcaactatcaactgccgagccagcgagagcgtcgataattacggcatccccttcatgaactggtatcagcagaagccaggacagccgcccaagctgcttatctacgccgcttccaaccggggatcaggggtgcccgatcgatttagtggaagcggtagtgggaccgatttcacactgaccatcagctcccttcaggccgaggatgtggctgtctattattgtcagcaatccgaggaagtgccgctcacgtttggtcagggaaccaaactggagatcaagcggaccgtagcggcgcctagtgtcttcatcttcccaccctccgacgaacagctgaagtctggcactgcttccgtcgtgtgcctgctcaacaacttttaccctagagaggcaaaagttcaatggaaagtagacaatgccttgcagtccgggaactcccaggagtctgtcacagagcaggatagtaaggactcaacctacagcctgtccagcacactgaccctctccaaagccgactacgagaagcacaaagtgtacgcttgcgaagttacgcatcaggggctgtcctcacccgttacaaaaagttttaacagaggggagtgc

SEQ ID NO: 27 - protein, 122 aa, synthetic construct
QVQLVQSGAEVKKPGSSVKVSCKASGYALSNYLIEWVRQAPGQGLEWMGVITPGSGTINYAQKFQGRVTITADESTSTVYMELSSLRSEDTAVYYCARSRWDPLYYYALEYWGQGTTVTVSS

SEQ ID NO: 28 - protein, 467 aa, synthetic construct
MDWTWRILFLVAAATGAHSQVQLVQSGAEVKKPGSSVKVSCKASGYALSNYLIEWVRQAPGQGLEWMGVITPGSGTINYAQKFQGRVTITADESTSTAYMELSSLRSEDTAVYYCARSRWDPLYYYALEYWGQGTTVTVSSASTKGPSVFPLAPCSRSTSESTAALGCLVKDYFPEPVTVSWNSGALTSGVHTFPAVLQSSGLYSLSSVVTVPSSNFGTQTYTCNVDHKPSNTKVDKTVERKCCVECPPCPAPPVAGPSVFLFPPKPKDTLMISRTPEVTCVVVDVSHEDPEVQFNWYVDGVEVHNAKTKPREEQFNSTFRVVSVLTVVHQDWLNGKEYKCKVSNKGLPAPIEKTISKTKGQPREPQVYTLPPSREEMTKNQVSLTCLVKGFYPSDIAVEWESNGQPENNYKTTPPMLDSDGSFFLYSKLTVDKSRWQQGNVFSCSVMHEALHNHYTQKSLSLSPGK

SEQ ID NO: 29 - protein, 15 aa, synthetic construct
GGGGSGGGGSGGGGS

SEQ ID NO: 30 - protein, 5 aa, synthetic construct
DKTHT

SEQ ID NO: 31 - protein, 10 aa, synthetic construct
GYVLPNYLIE

SEQ ID NO: 32 - protein, 10 aa, synthetic construct
VTTPGGGTIN

SEQ ID NO: 33 - protein, 13 aa, synthetic construct
SRWDPLYYYALEY

SEQ ID NO: 34 - protein, 15 aa, synthetic construct
RASESVDNYGIPFMN

SEQ ID NO: 35 - protein, 7 aa, synthetic construct
AASNRGS

SEQ ID NO: 36 - protein, 9 aa, synthetic construct
QQSEEVPLT

SEQ ID NO: 37 - protein, 122 aa, synthetic construct
QVQLVQSGAEVKKPGSSVKVSCKASGYVLPNYLIEWVRQAPGQGLEWMGVTTPGGGTINYAQKFQGRVTITADESTSTAYMELSSLRSEDTAVYYCARSRWDPLYYYALEYWGQGTTVTVSS

SEQ ID NO: 38 - protein, 114 aa, synthetic construct; identical to SEQ ID NO: 18

SEQ ID NO: 39 - protein, 230 aa, synthetic construct
QVQLVQSGAEVKKPGSSVKVSCKASGYVLPNYLIEWVRQAPGQGLEWMGVTTPGGGTINYAQKFQGRVTITADESTSTAYMELSSLRSEDTAVYYCARSRWDPLYYYALEYWGQGTTVTVSSASTKGPSVFPLAPSSKSTSGGTAALGCLVKDYFPEPVTVSWNSGALTSGVHTFPAVLQSSGLYSLSSVVTVPSSSLGTQTYICNVNHKPSNTKVDKKVEPKSCDKTHT

SEQ ID NO: 40 - DNA, 690 bp, synthetic construct
  source 1..690: mol_type = other DNA
caagtgcagctggtgcagtcaggggccgaggttaagaagccagggagcagcgtcaaggtatcttgtaaagcgtctggttacgtccttccaaactacctgatcgaatgggtgaggcaggctcccggccaaggcctggaatggatgggagttaccacccctgggggcggcaccattaattacgcccagaaatttcagggacgagtgacgattaccgccgacgagtccaccagtactgcctacatggagctgtcctcactccgcagcgaggacacggcagtttactactgcgcccggagtcgatgggaccctctttactattatgctctggaatactggggccagggaacgaccgttacagtgtcatctgctagcacaaaaggaccatcagtcttcccacttgctccttcatctaagagcacaagtggtggcactgcagcccttggctgcctggtgaaagattatttccccgaacctgttacagtttcttggaactccggtgcactgacatccggagtacacactttcccagctgtgctgcagagctcaggactgtatagcctgtcttcggtggtcactgttccatcgtcgagtcttggcacacagacatatatttgcaacgtcaatcacaagccctccaacacaaaagtggataagaaggtcgagcccaaatcttgtgacaaaacacacaca

SEQ ID NO: 41 - protein, 448 aa, synthetic construct
QVQLVQSGAEVKKPGSSVKVSCKASGYVLPNYLIEWVRQAPGQGLEWMGVTTPGGGTINYAQKFQGRVTITADESTSTAYMELSSLRSEDTAVYYCARSRWDPLYYYALEYWGQGTTVTVSSASTKGPSVFPLAPCSRSTSESTAALGCLVKDYFPEPVTVSWNSGALTSGVHTFPAVLQSSGLYSLSSVVTVPSSNFGTQTYTCNVDHKPSNTKVDKTVERKCCVECPPCPAPPVAGPSVFLFPPKPKDTLMISRTPEVTCVVVDVSHEDPEVQFNWYVDGVEVHNAKTKPREEQFNSTFRVVSVLTVVHQDWLNGKEYKCKVSNKGLPAPIEKTISKTKGQPREPQVYTLPPSREEMTKNQVSLTCLVKGFYPSDIAVEWESNGQPENNYKTTPPMLDSDGSFFLYSKLTVDKSRWQQGNVFSCSVMHEALHNHYTQKSLSLSPGK

SEQ ID NO: 42 - protein, 218 aa, synthetic construct; identical to SEQ ID NO: 2

SEQ ID NO: 43 - DNA, 1344 bp, synthetic construct
  source 1..1344: mol_type = other DNA
caagtgcagctggtgcagtcaggggccgaggttaagaagccagggagcagcgtcaaggtatcttgtaaagcgtctggttacgtccttccaaactacctgatcgaatgggtgaggcaggctcccggccaaggcctggaatggatgggagttaccacccctgggggcggcaccattaattacgcccagaaatttcagggacgagtgacgattaccgccgacgagtccaccagtactgcctacatggagctgtcctcactccgcagcgaggacacggcagtttactactgcgcccggagtcgatgggaccctctttactattatgctctggaatactggggccagggaacgaccgttacagtgtcatctgctagcaccaagggcccatcggtcttccccctggcgccctgctccaggagcacctccgagagcacagcggccctgggctgcctggtcaaggactacttccccgaaccggtgacggtgtcgtggaactcaggcgctctgaccagcggcgtgcacaccttcccggctgtcctacagtcctcaggactctactccctcagcagcgtggtgaccgtgccctccagcaacttcggcacccagacctacacctgcaacgtagatcacaagcccagcaacaccaaggtggacaagacagttgagcgcaaatgttgtgtcgagtgcccaccgtgcccagcaccacctgtggcaggaccgtcagtcttcctcttccccccaaaacccaaggacaccctcatgatctcccggacccctgaggtcacgtgcgtggtggtggacgtgagccacgaagaccccgaggtccagttcaactggtacgtggacggcgtggaggtgcataatgccaagacaaagccacgggaggagcagttcaacagcacgttccgtgtggtcagcgtcctcaccgtcgtgcaccaggactggctgaacggcaaggagtacaagtgcaaggtctccaacaaaggcctcccagcccccatcgagaaaaccatctccaaaaccaaagggcagccccgagaaccacaggtgtacaccctgcccccatcccgggaggagatgaccaagaaccaggtcagcctgacctgcctggtcaaaggcttctaccccagcgacatcgccgtggagtgggagagcaatgggcagccggagaacaactacaagaccacacctcccatgctggactccgacggctccttcttcctctacagcaagctcaccgtggacaagagcaggtggcagcaggggaacgtcttctcatgctccgtgatgcatgaggctctgcacaaccactacacgcagaagagcctctccctgtctccgggtaaa

SEQ ID NO: 44 - DNA, 654 bp, synthetic construct; identical to SEQ ID NO: 26
  source 1..654: mol_type = other DNA

SEQ ID NO: 45 - protein, 10 aa, synthetic construct
  MOD_RES 3: note = Any amino acid except Ala
  MOD_RES 5: note = Any amino acid except Ser
GYXLXNYLIE

SEQ ID NO: 46 - protein, 10 aa, synthetic construct
  MOD_RES 2: note = Any amino acid except Ile
  MOD_RES 6: note = Any amino acid except Ser
VXTPGXGTIN

SEQ ID NO: 47 - protein, 448 aa, synthetic construct
QVQLVQSGAEVKKPGSSVKVSCKASGYVLPNYLIEWVRQAPGQGLEWMGVTTPGGGTINYAQKFQGRVTITADESTSTAYMELSSLRSEDTAVYYCARSRWDPLYYYALEYWGQGTTVTVSSASTKGPSVFPLAPCSRSTSESTAALGCLVKDYFPEPVTVSWNSGALTSGVHTFPAVLQSSGLYSLSSVVTVPSSNFGTQTYTCNVDHKPSNTKVDKTVERKCCVECPPCPAPPVAGPSVFLFPPKPKDTLMISRTPEVTCVVVDVSHEDPEVQFNWYVDGVEVHNAKTKPREEQFNSTFRVVSVLTVVAQDWLNGKEYKCKVSNKGLPAPIEKTISKTKGQPREPQVYTLPPSREEMTKNQVSLTCLVKGFYPSDIAVEWESNGQPENNYKTTPPMLDSDGSFFLYSKLTVDKSRWQQGNVFSCSVMHEALHNHYTQKSLSLSPGK

SEQ ID NO: 48 - DNA, 1344 bp, synthetic construct
  source 1..1344: mol_type = other DNA
caagtgcagctggtgcagtcaggggccgaggttaagaagccagggagcagcgtcaaggtatcttgtaaagcgtctggttacgtccttccaaactacctgatcgaatgggtgaggcaggctcccggccaaggcctggaatggatgggagttaccacccctgggggcggcaccattaattacgcccagaaatttcagggacgagtgacgattaccgccgacgagtccaccagtactgcctacatggagctgtcctcactccgcagcgaggacacggcagtttactactgcgcccggagtcgatgggaccctctttactattatgctctggaatactggggccagggaacgaccgttacagtgtcatctgctagcaccaagggcccatcggtcttccccctggcgccctgctccaggagcacctccgagagcacagcggccctgggctgcctggtcaaggactacttccccgaaccggtgacggtgtcgtggaactcaggcgctctgaccagcggcgtgcacaccttcccggctgtcctacagtcctcaggactctactccctcagcagcgtggtgaccgtgccctccagcaacttcggcacccagacctacacctgcaacgtagatcacaagcccagcaacaccaaggtggacaagacagttgagcgcaaatgttgtgtcgagtgcccaccgtgcccagcaccacctgtggcaggaccgtcagtcttcctcttccccccaaaacccaaggacaccctcatgatctcccggacccctgaggtcacgtgcgtggtggtggacgtgagccacgaagaccccgaggtccagttcaactggtacgtggacggcgtggaggtgcataatgccaagacaaagccacgggaggagcagttcaacagcacgttccgtgtggtcagcgtcctcaccgtcgtggcccaggactggctgaacggcaaggagtacaagtgcaaggtctccaacaaaggcctcccagcccccatcgagaaaaccatctccaaaaccaaagggcagccccgagaaccacaggtgtacaccctgcccccatcccgggaggagatgaccaagaaccaggtcagcctgacctgcctggtcaaaggcttctaccccagcgacatcgccgtggagtgggagagcaatgggcagccggagaacaactacaagaccacacctcccatgctggactccgacggctccttcttcctctacagcaagctcaccgtggacaagagcaggtggcagcaggggaacgtcttctcatgctccgtgatgcatgaggctctgcacaaccactacacgcagaagagcctctccctgtctccgggtaaa

SEQ ID NO: 49 - protein, 19 aa, synthetic construct
MDWTWRILFLVAAATGAHS

SEQ ID NO: 50 - protein, 227 aa, Homo sapiens
DKTHTCPPCPAPELLGGPSVFLFPPKPKDTLMISRTPEVTCVVVDVSHEDPEVKFNWYVDGVEVHNAKTKPREEQYNSTYRVVSVLTVLHQDWLNGKEYKCKVSNKALPAPIEKTISKAKGQPREPQVYTLPPSRDELTKNQVSLTCLVKGFYPSDIAVEWESNGQPENNYKTTPPVLDSDGSFFLYSKLTVDKSRWQQGNVFSCSVMHEALHNHYTQKSLSLSPGK

SEQ ID NO: 51 - protein, 223 aa, Homo sapiens
VECPPCPAPPVAGPSVFLFPPKPKDTLMISRTPEVTCVVVDVSHEDPEVQFNWYVDGVEVHNAKTKPREEQFNSTFRVVSVLTVVHQDWLNGKEYKCKVSNKGLPAPIEKTISKTKGQPREPQVYTLPPSREEMTKNQVSLTCLVKGFYPSDIAVEWESNGQPENNYKTTPPMLDSDGSFFLYSKLTVDKSRWQQGNVFSCSVMHEALHNHYTQKSLSLSPGK

SEQ ID NO: 52 - protein, 251 aa, synthetic construct
QVQLVQSGAEVKKPGSSVKVSCKASGYVLPNYLIEWVRQAPGQGLEWMGVTTPGGGTINYAQKFQGRVTITADESTSTAYMELSSLRSEDTAVYYCARSRWDPLYYYALEYWGQGTTVTVSSGGGGSGGGGSGGGGSDIVMTQSPDSLAVSLGERATINCRASESVDNYGIPFMNWYQQKPGQPPKLLIYAASNRGSGVPDRFSGSGSGTDFTLTISSLQAEDVAVYYCQQSEEVPLTFGQGTKLEIKRTV

SEQ ID NO: 53 - protein, 251 aa, synthetic construct
DIVMTQSPDSLAVSLGERATINCRASESVDNYGIPFMNWYQQKPGQPPKLLIYAASNRGSGVPDRFSGSGSGTDFTLTISSLQAEDVAVYYCQQSEEVPLTFGQGTKLEIKRTVGGGGSGGGGSGGGGSQVQLVQSGAEVKKPGSSVKVSCKASGYVLPNYLIEWVRQAPGQGLEWMGVTTPGGGTINYAQKFQGRVTITADESTSTAYMELSSLRSEDTAVYYCARSRWDPLYYYALEYWGQGTTVTVSS

SEQ ID NO: 54 - protein, 223 aa, synthetic construct
QVQLVQSGAEVKKPGSSVKVSCKASGYVLPNYLIEWVRQAPGQGLEWMGVTTPGGGTINYAQKFQGRVTITADESTSTAYMELSSLRSEDTAVYYCARSRWDPLYYYALEYWGQGTTVTVSSASTKGPSVFPLAPCSRSTSESTAALGCLVKDYFPEPVTVSWNSGALTSGVHTFPAVLQSSGLYSLSSVVTVPSSNFGTQTYTCNVDHKPSNTKVDKTVERK